European Patent Application EP 4 703 383 A1, published March 4, 2026. Title: PROLACTIN RECEPTOR ANTIBODY AND USE THEREOF. Applicant: Shenzhen Genuine Biomedical Technology Co., LTD. The sequence listing filed with the application follows.

SEQUENCE LISTING (102 sequences)

SEQ ID NO: 1 - protein, 120 aa, synthetic construct
QVQLQQPGSELVRPGASVRLSCKASGFTFTTYWVHWVKQRPGQGLEWIGNISPGSGSTNYDEKFKSKASLTVDTFSNTAYMQLSSLTSEDSAVYYCIRHSGNYFNAMDYWGQGTSVTVSS

SEQ ID NO: 2 - protein, 120 aa, synthetic construct
QVQLQQPGSELVRPGASVKLSCKASGFTFTTYWVHWVKQRPGQGLEWIGNISPGGGSTNYDEKFKSKASLTVDTFSNTAYMQLSSLTSEDSAVYYCIRHSGNYFNAMDYWGQGTTVTVSS

SEQ ID NO: 3 - protein, 120 aa, synthetic construct
QVQLQQPGSELVRPGASVKLSCKASGFTFTTFWVHWVKQRPGQGLEWIGNISPGSTSTNYNEKFKNKASLTVDTFSNTAYMQLSSLTSEDSAVYYCIRHSGNYFNAMDYWGQGTSVTVSS

SEQ ID NO: 4 - protein, 120 aa, synthetic construct
QVQLQQPGSELVRPGASVKLSCKASGFTFTTYWVHWVKQRPGQGLEWIGNISPGSGSTNYDEKFKSKASLTVDTFSNTAYMQLSSLTSEDSAVYYCIRHSGNYFNAMDYWGQGTSVTVSS

SEQ ID NO: 5 - protein, 116 aa, synthetic construct
EVQLQQSGAELVRPGTSVQISCKASGYTFTNNWLAWIKQRPGHGLEWIGDIYPGGVYTNYNEKFKGKATLTADTSSSTAYMQLSSLTSEDSAVYFCYYGDFWSAYWGQGTLVTVSA

SEQ ID NO: 6 - protein, 120 aa, synthetic construct
QVQLQQPGSELVRPGASVKLSCKASGFTFTTYWVHWVKQRPGQGLEWIGNISPGSGSTNYDEKFKSKASLTVDTFSNTAYMQLSSLTSEDSAVYYCIRHSGNYFNAMDYWGQGTTVTVSS

SEQ ID NO: 7 - protein, 120 aa, synthetic construct
QVQLQQPGSELVRPGASVKLSCKASGFTFATYWVHWVKQRPGQGLEWIGNISPGSVSTNYDEKFKSKASLTVDTFSNTAYMQLSSLTSEDSAVYYCIRHSGNYFNAMDYWGQGTTLTVSS

SEQ ID NO: 8 - protein, 120 aa, synthetic construct
QVQLQQPGSELVRPGASVKLSCKASGFTFTTYWVHWVKQRPGQGLEWIGNISPGGGSTNYDEKFKSKASLTVDTFSNTAYMQLGSLTSEDSAVYYCIRHSGNYFNAMDYWGQGTTLTVSS

SEQ ID NO: 9 - protein, 118 aa, synthetic construct
QVQLQQPGSELVRPGASVKLSCKASGYTFTSYWMHWVKQRPGQGLEWIGNIYPGSGSTNYDEKFKSKATLTVDTSSSTAYMQLSSLTSEDSAVYYCTRGNYRYYFDYWGQGTTLTVSS

SEQ ID NO: 10 - protein, 120 aa, synthetic construct
QVQLQQPGSELVRPGASVKLSCKASGFTFTTFWVHWVKQRPGQGLEWIGNISPGGTSTNYDEKFKSKASLTVDTFSNTAYMQLSSLTSEDSAVYYCIRHSGNYFNAMDYWGQGTSVTVSS

SEQ ID NO: 11 - protein, 120 aa, synthetic construct
QVQLQQPGSELVRPGASVKLSCKASGFTFTTYWVHWVKQRPGQGLEWIGNISPGSGSTNYDEKFKSKASLTVDTFSNTAYMQLSSLTSEDSAVYYCIRHSGNYFNAMDYWGQGTTLTVSS

SEQ ID NO: 12 - protein, 120 aa, synthetic construct
QVQLQQPGSELVRPGASVKLSCKASGFTFTTFWVHWVKQRPGQGLEWIGNISPGSTSTNYNEKFKNKASLTVDTFSNTAYMQLSSLTSEDSAVYYCIRHSGNYFNAMDYWGQGTTLTVSS

SEQ ID NO: 13 - protein, 120 aa, synthetic construct
QVQLKESGPGLVAPSQSLSITCTVSGFSLTGFGVNWFRQPPGRGLEWLGMIWGDGSTDYNSALKSRLSISKDNSKSQVFLKMNSLQTDDTARYYCARVLYYYGGNSFAYWGQGTLVTVSA

SEQ ID NO: 14 - protein, 123 aa, synthetic construct
DVKLVESGGGLVKPGGSLKLACAASGFTFSSYTMSWVRQTPEKRLEWVATISSGGSYTYYPDSVKGRFTISRDNAKNTLYLQLSSLKSEDTAMYYCTRDRYYSTTPDWYFDVWGAGTTVTVSS

SEQ ID NO: 15 - protein, 120 aa, synthetic construct
QVQLQQSGPGLVAPSQSLSITCTVSGFSLTSYGVNWVRQPPGKGLEWLGIIGAGGSTNYNSALMSRLSISKDNSKSQVFLKMNSLQTDDTAMYYCARSLYYYGSSSFAYWGQGTLVTVSA

SEQ ID NO: 16 - protein, 118 aa, synthetic construct
EVMLVESGGGLVQPGGSRKLSCAASGFTFSSFGMNWVRQAPEKGLEWVAYISSGSSIIYYADTVKGRFTISRDNPKNTLFLQMTSLRSEDTAMYYCTRFYGYIPFDYWGQGTTLTVSS

SEQ ID NO: 17 - protein, 123 aa, synthetic construct
EVMLVESGGGLVKPGGSLKLACAASGFTFSSYTMSWVRQTPEKRLEWVATISSGGSYTYYPDSVKGRFTISRDNAKNTLYLQLSSLKSEDTAMYYCTRDRYYSTTPDWYFDVWGAGTTLTVSS

SEQ ID NO: 18 - protein, 116 aa, synthetic construct
DVHLVESGPGLVKPSQSLSLTCTVTGYSITSDYAWNWIRQFPGNKLEWMGYISYSGSTGYSPSLKSRVSITRDTSKNQFFLQLNSVTTEDTATYFCARNNWAFDFWGQGTTLTVSS

SEQ ID NO: 19 - protein, 120 aa, synthetic construct
EVHLVESGPDLVKPSQSLSLTCTVTGYSITSGYNWHWIRQFPGNKLEWMGYIHYSGSTKYDPSLKSRISFTRDTSRNQFFLQLNSVTTEDRATYYCARSEAGGYSWFAYWGQGTLVTVSA

SEQ ID NO: 20 - protein, 120 aa, synthetic construct
EVQLVQSGAEVKKPGASVKVSCKASGFTFTTFWVHWVRQAPGQGLEWIGNISPGSTSTNYAQKFQGRATLTVDTSISTAYMELSSLRSEDTAVYYCIRHSGNYFNAMDYWGQGTLVTVSS

SEQ ID NO: 21 - protein, 120 aa, synthetic construct
EVQLVQSGAEVKKPGASVKVSCKASGFTFTTFWVHWVRQAPGQGLEWIGNIAPGSTSTNYAQKFQGRATLTVDTSISTAYMELSSLRSEDTAVYYCIRHSGNYFNAMDYWGQGTLVTVSS

SEQ ID NO: 22 - protein, 116 aa, synthetic construct
EVQLVQSGAEVKKPGSSVKVSCKASGYTFTNNWLAWIRQAPGQGLEWIGDIYPGGVYTNYNQKFQGRATLTADTSTSTAYMELSSLRSEDTAVYFCYYGDFWSAYWGQGTLVTVSS

SEQ ID NO: 23 - protein, 118 aa, synthetic construct
EVQLVESGGGLVQPGGSLRLSCAASGFTFSSFGMNWVRQAPGKGLEWVAYISSGSSIIYYADSVKGRFTISRDNSKNTLYLQMNSLRAEDTAVYYCTRFYGYIPFDYWGQGTLVTVSS

SEQ ID NO: 24 - protein, 112 aa, synthetic construct
DIVMTQATPSVPVAPGESVSISCRSSKSLLHTNGYTYLYWFLQRPGQSPQLLIYRMSNLASGVPDRFSGSGSGTAFTLRISRVEAEDVGVYYCMQHLEYPLTFGAGTKLELK

SEQ ID NO: 25 - protein, 112 aa, synthetic construct
DIVMTQAAPSVPVTPGESVSISCRSSKSLLHSNGNTYLYWFLQRPGQSPQLLIYRMSNLASGVPDRFSGSGSGTAFTLRISRVEAEDVGVYYCMQHLEYPFTFGSGTKLEIK

SEQ ID NO: 26 - protein, 112 aa, synthetic construct
DIVMTQAAPSVPVTPGESVSISCRSSKSLLHSNGNTYLYWFLQRPGQSPQLLIYRMSNLASGVPDRFSGSGSGTAFTLRISRVEAEDVGIYYCMQHLEYPLTFGAGTKLELK

SEQ ID NO: 27 - protein, 112 aa, synthetic construct
DIVMTQAAPSVFVTPGESVSISCRSSKSLLHSNGNTYLYWFLQRPGQSPQLLIYQMSNRASGVPDRLSGSGSGTAFTLRISRVEAEDVGVYYCMQHLEYPFTFGGGTKLEIK

SEQ ID NO: 28 - protein, 112 aa, synthetic construct
DIVMTQAAPSVPVTPGESVSISCRSSKSLLHSNGNTYLYWFLQRPGQSPQLLIYRMSNLASGVPDRFSGSGSGTAFTLRISRVEAEDVGVYYCMQHLEYPLTFGAGTKLELK

SEQ ID NO: 29 - protein, 112 aa, synthetic construct
DIVMTQAAPSVLVTPGESVSISCRSSKSLLHSNGNTYLYWFLQRPGQSPQLVIYRMSNLASGVPDRFSGSGSGTAFTLRISRVEAEDVGVYYCMQHLEYPFTFGAGTKLELK

SEQ ID NO: 30 - protein, 111 aa, synthetic construct
DIVLTQSPASLAVSLGQRATISCRASESVDKSGFSFMNWFQQKPGQPPKLLIYAASNRGSGVPARFSGSGSGTDFSLNIHPMEEDDTAMYFCQQSKEVPWTFGGGTKLEIK

SEQ ID NO: 31 - protein, 112 aa, synthetic construct
DIVMTQAAPSVPVTPGESVSISCRSSKSLLHSNGNTYLYWFLQRPGQSPQLLIYRMSNLASGVPDRFSGSGSGTAFTLRISRVEAEDVGVYYCMQHLEYPFTFGGGTKLEIK

SEQ ID NO: 32 - protein, 112 aa, synthetic construct
DIVMTQAAPSVPVTPGESVTISCRSSKSLLHSNGKTYLYWFLQRPGQSPQLLIYWMSNLASGVPDRFSGSGSGTAFTLRISRVEAEDVGVYYCMQHLEYPFTFGVGTKLELK

SEQ ID NO: 33 - protein, 112 aa, synthetic construct
DVLMTQTPLSLPVSLGDQASISCRSSQSIVHSNGNTYLEWYLQKPGQSPKLLIYKVSSRFSGVPDRFSGSGSGTDFTLKISRVEAEDLGVYYCFQGSHVPYTFGGGTKLEIK

SEQ ID NO: 34 - protein, 107 aa, synthetic construct
DIVLTQSPATLSVTPGDSVSLSCRATQIIFNNLHWYQQKSHESPRLLITYTSQSISGIPSRFSGSGSGTDFTLTINSVETEDFGMYFCQQSNTWPRTFGGGTKLEIK

SEQ ID NO: 35 - protein, 112 aa, synthetic construct
DIVMTQTPLSLPVSLGDQASISCRSSQSIVHSNGNTYLEWYLQKPGQSPKLLIYKVSNRFSGVPDRFSGSGSGTDFTLKISRVEAEDLGVYYCFQGSHVPWTFGGGTKLELK

SEQ ID NO: 36 - protein, 106 aa, synthetic construct
DIVMTQSPAIMSASPGEKVTMTCSASSSLIYMHWYQQKSSTSPKLWIYDTSKLASGVPGRFSGSGSGNSYSLTTSSMEAEDVATYYCFQGSGYPLTFGGGTKLEIK

SEQ ID NO: 37 - protein, 107 aa, synthetic construct
DIVITQSPATLSVTPGDSVSLSCRATQIIFNNLHWYQQKSHESPRLLITYTSQSISGIPSRFSGSGSGTDFTLTINSVETEDFGMYFCQQSNTWPRTFGGGTKLEIK

SEQ ID NO: 38 - protein, 106 aa, synthetic construct
DIVLTQSPAIMSASPGEKVTMTCSASSSVNYMHWYQQKSGTSPKRWIYDTSKLASGVPARFSGSGSGTSYSLTISSMEAEDAATYYCQQWSSNPLTFGAGTKLELK

SEQ ID NO: 39 - protein, 106 aa, synthetic construct
DIVMTQSPAIMSASPGEKVTMACSASSSVNYMHWYQQKSGTSPKRWIYDTSKLASGVPARFSGSGSGTSYSLTISSMEAEDAATYYCQQWSSNPLTFGAGTKLELK

SEQ ID NO: 40 - protein, 112 aa, synthetic construct
DIVMTQSPLSLPVTPGEPASISCRSSKSLLHSNGNTYLYWFLQKPGQSPQLLIYRMSNRASGVPDRFSGSGSGTDFTLKISRVEAEDVGVYYCMQHLEYPLTFGQGTKVEIK

SEQ ID NO: 41 - protein, 106 aa, synthetic construct
DIQMTQSPSSLSASVGDRVTITCRASSSLIYLHWYQQKPGKAPKLWIYDTSKLASGVPSRFSGSGSGNDYTLTISSLQPEDFATYYCFQGSGYPLTFGQGTKVEIK

SEQ ID NO: 42 - protein, 8 aa, synthetic construct
GFTFTTYW

SEQ ID NO: 43 - protein, 8 aa, synthetic construct
GFTFTTFW

SEQ ID NO: 44 - protein, 8 aa, synthetic construct
GYTFTNNW

SEQ ID NO: 45 - protein, 8 aa, synthetic construct
GFTFATYW

SEQ ID NO: 46 - protein, 8 aa, synthetic construct
GYTFTSYW

SEQ ID NO: 47 - protein, 8 aa, synthetic construct
GFSLTGFG

SEQ ID NO: 48 - protein, 8 aa, synthetic construct
GFTFSSYT

SEQ ID NO: 49 - protein, 8 aa, synthetic construct
GFSLTSYG

SEQ ID NO: 50 - protein, 8 aa, synthetic construct
GFTFSSFG

SEQ ID NO: 51 - protein, 9 aa, synthetic construct
GYSITSDYA

SEQ ID NO: 52 - protein, 9 aa, synthetic construct
GYSITSGYN

SEQ ID NO: 53 - protein, 8 aa, synthetic construct
ISPGSGST

SEQ ID NO: 54 - protein, 8 aa, synthetic construct
ISPGGGST

SEQ ID NO: 55 - protein, 8 aa, synthetic construct
ISPGSTST

SEQ ID NO: 56 - protein, 8 aa, synthetic construct
IYPGGVYT

SEQ ID NO: 57 - protein, 8 aa, synthetic construct
ISPGSVST

SEQ ID NO: 58 - protein, 8 aa, synthetic construct
IYPGSGST

SEQ ID NO: 59 - protein, 8 aa, synthetic construct
ISPGGTST

SEQ ID NO: 60 - protein, 7 aa, synthetic construct
IWGDGST

SEQ ID NO: 61 - protein, 8 aa, synthetic construct
ISSGGSYT

SEQ ID NO: 62 - protein, 7 aa, synthetic construct
IGAGGST

SEQ ID NO: 63 - protein, 8 aa, synthetic construct
ISSGSSII

SEQ ID NO: 64 - protein, 7 aa, synthetic construct
ISYSGST

SEQ ID NO: 65 - protein, 7 aa, synthetic construct
IHYSGST

SEQ ID NO: 66 - protein, 8 aa, synthetic construct
IAPGSTST

SEQ ID NO: 67 - protein, 13 aa, synthetic construct
IRHSGNYFNAMDY

SEQ ID NO: 68 - protein, 9 aa, synthetic construct
YYGDFWSAY

SEQ ID NO: 69 - protein, 11 aa, synthetic construct
TRGNYRYYFDY

SEQ ID NO: 70 - protein, 14 aa, synthetic construct
ARVLYYYGGNSFAY

SEQ ID NO: 71 - protein, 16 aa, synthetic construct
TRDRYYSTTPDWYFDV

SEQ ID NO: 72 - protein, 14 aa, synthetic construct
ARSLYYYGSSSFAY

SEQ ID NO: 73 - protein, 11 aa, synthetic construct
TRFYGYIPFDY

SEQ ID NO: 74 - protein, 9 aa, synthetic construct
ARNNWAFDF

SEQ ID NO: 75 - protein, 13 aa, synthetic construct
ARSEAGGYSWFAY

SEQ ID NO: 76 - protein, 11 aa, synthetic construct
KSLLHTNGYTY

SEQ ID NO: 77 - protein, 11 aa, synthetic construct
KSLLHSNGNTY

SEQ ID NO: 78 - protein, 10 aa, synthetic construct
ESVDKSGFSF

SEQ ID NO: 79 - protein, 11 aa, synthetic construct
KSLLHSNGKTY

SEQ ID NO: 80 - protein, 11 aa, synthetic construct
QSIVHSNGNTY

SEQ ID NO: 81 - protein, 6 aa, synthetic construct
QIIFNN

SEQ ID NO: 82 - protein, 5 aa, synthetic construct
SSLIY

SEQ ID NO: 83 - protein, 5 aa, synthetic construct
SSVNY

SEQ ID NO: 84-90 - skipped (7 entries)

SEQ ID NO: 91 - protein, 9 aa, synthetic construct
MQHLEYPLT

SEQ ID NO: 92 - protein, 9 aa, synthetic construct
MQHLEYPFT

SEQ ID NO: 93 - protein, 9 aa, synthetic construct
QQSKEVPWT

SEQ ID NO: 94 - protein, 9 aa, synthetic construct
FQGSHVPYT

SEQ ID NO: 95 - protein, 9 aa, synthetic construct
QQSNTWPRT

SEQ ID NO: 96 - protein, 9 aa, synthetic construct
FQGSHVPWT

SEQ ID NO: 97 - protein, 9 aa, synthetic construct
FQGSGYPLT

SEQ ID NO: 98 - protein, 9 aa, synthetic construct
QQWSSNPLT

SEQ ID NO: 99 - protein, 231 aa, synthetic construct
QLPPGKPEIFKCRSPNKETFTCWWRPGTDGGLPTNYSLTYHREGETLMHECPDYITGGPNSCHFGKQYTSMWRTYIMMVNATNQMGSSFSDELYVDVTYIVQPDPPLELAVEVKQPEDRKPYLWIKWSPPTLIDLKTGWFTLLYEIRLKPEKAAEWEIHFAGQQTEFKILSLHPGQKYLVQVRCKPDHGYWSAWSPATFIQIPSDFTMNDGLNDIFEAQKIEWHEHHHHHH

SEQ ID NO: 100 - protein, 446 aa, synthetic construct
QLPPGKPEIFKCRSPNKETFTCWWRPGTDGGLPTNYSLTYHREGETLMHECPDYITGGPNSCHFGKQYTSMWRTYIMMVNATNQMGSSFSDELYVDVTYIVQPDPPLELAVEVKQPEDRKPYLWIKWSPPTLIDLKTGWFTLLYEIRLKPEKAAEWEIHFAGQQTEFKILSLHPGQKYLVQVRCKPDHGYWSAWSPATFIQIPSDFTMNDGSGEPRGPTIKPCPPCKCPAPNLLGGPSVFIFPPKIKDVLMISLSPIVTCVVVDVSEDDPDVQISWFVNNVEVHTAQTQTHREDYNSTLRVVSALPIQHQDWMSGKEFKCKVNNKDLPAPIERTISKPKGSVRAPQVYVLPPPEEEMTKKQVTLTCMVTDFMPEDIYVEWTNNGKTELNYKNTEPVLDSDGSYFMYSKLRVEKKNWVERNSYSCSVVHEGLHNHHTTKSFSRTPGK

SEQ ID NO: 101 - protein, 231 aa, synthetic construct
QLPPGKPEIFKCRSPNKETFTCWWRPGTDGGLPTNYSLTYHREGETLMHECPDYITGGPNSCHFGKQYTSMWRTYVMMVNATNQMGSSFSDELYVDVTYIVQPDPPLELTVEVKQPEDRKPYLWMKWSPPTLIDLKTGWFTLLYEIRLKPEKAAEWETHFAGQQTEFKILSLHPGQKYLVQVRCKPDHGYWSAWSPATFIQIPSDFIMNDGLNDIFEAQKIEWHEHHHHHH

SEQ ID NO: 102 - protein, 882 aa, synthetic construct
MKENVASATVFTLLLFLNTCLLNGQLPPGKPEIFKCRSPNKETFTCWWRPGTDGGLPTNYSLTYHREGETLMHECPDYITGGPNSCHFGKQYTSMWRTYIMMVNATNQMGSSFSDELYVDVTYIVQPDPPLELAVEVKQPEDRKPYLWIKWSPPTLIDLKTGWFTLLYEIRLKPEKAAEWEIHFAGQQTEFKILSLHPGQKYLVQVRCKPDHGYWSAWSPATFIQIPSDFTMNDTTVWISVAVLSAVICLIIVWAVALKGYSMVTCIFPPVPGPKIKGFDAHLLEKGKSEELLSALGCQDFPPTSDYEDLLVEYLEVDDSEDQHLMSVHSKEHPSQGMKPTYLDPDTDSGRGSCDSPSLLSEKCEEPQANPSTFYDPEVIEKPENPETTHTWDPQCISMEGKIPYFHAGGSKCSTWPLPQPSQHNPRSSYHNITDVCELAVGPAGAPATLLNEAGKDALKSSQTIKSREEGKATQQREVESFHSETDQDTPWLLPQEKTPFGSAKPLDYVEIHKVNKDGALSLLPKQRENSGKPKKPGTPENNKEYAKVSGVMDNNILVLVPDPHAKNVACFEESAKEAPPSLEQNQAEKALANFTATSSKCRLQLGGLDYLDPACFTHSFHVDATNFSLLKQAGDVEENPGPMVSKGEELFTGVVPILVELDGDVNGHKFSVSGEGEGDATYGKLTLKFICTTGKLPVPWPTLVTTLTYGVQCFSRYPDHMKQHDFFKSAMPEGYVQERTIFFKDDGNYKTRAEVKFEGDTLVNRIELKGIDFKEDGNILGHKLEYNYNSHNVYIMADKQKNGIKVNFKIRHNIEDGSVQLADHYQQNTPIGDGPVLLPDNHYLSTQSALSKDPNEKRDHMVLLEFVTAAGITLGMDELYK